European Patent Specification EP 3 894 595 B1, published October 29, 2025. Title: Nucleic acid amplification and identification method. Applicant: LEXOGEN GMBH. The sequence listing filed with the application follows.

SEQUENCE LISTING (67 sequences)

SEQ ID NO: 1 - DNA, 41 bp, Artificial Sequence
  oligo
  modified_base 1: /mod_base="OTHER" /note="5' phosphorylated; a or g or c or t"
  misc_difference 2,3,4,5,6: /note="a or g or c or t"
  modified_base 41: /mod_base="OTHER" /note="3' Inverted dT (reverse linkage)"
nnnnnnagatcggaagagcacacgtctgaactccagtcacn

SEQ ID NO: 2 - DNA, 35 bp, Artificial Sequence
  oligo
  modified_base 1: /mod_base="OTHER" /note="5' phosphorylated; a or g or c or t"
  misc_difference 2,3,4,5,6,7,8,9,10: /note="a or g or c or t"
  modified_base 35: /mod_base="OTHER" /note="3' Inverted dT (reverse linkage)"
nnnnnnnnnnagatcggaagagcacacgtctgaan

SEQ ID NO: 3 - DNA, 43 bp, Artificial Sequence
  oligo
  modified_base 1: /mod_base="OTHER" /note="5' phosphorylated; a or g or c or t"
  misc_difference 2,3,4,5,6,7,8,9,10: /note="a or g or c or t"
  modified_base 43: /mod_base="OTHER" /note="3' Inverted dT (reverse linkage)"
nnnnnnnnnnagatcggaagagcgtcgtgtagggaaagagtgn

SEQ ID NO: 4 - DNA, 34 bp, Artificial Sequence
  oligo
  modified_base 1: /mod_base="OTHER" /note="5' phosphorylated; a or g or c or t"
  misc_difference 2,3,4,5,6,7,8,9,10: /note="a or g or c or t"
  modified_base 34: /mod_base="OTHER" /note="3' Inverted dT (reverse linkage)"
nnnnnnnnnnagatcggaagagcgtcgtgtaggn

SEQ ID NO: 5 - DNA, 44 bp, Artificial Sequence
  oligo
  modified_base 1: /mod_base="OTHER" /note="5' phosphorylated; a or g or c or t"
  misc_difference 2,3,4,5,6,7,8,9,10,11: /note="a or g or c or t"
  modified_base 44: /mod_base="OTHER" /note="3' Inverted dT (reverse linkage)"
nnnnnnnnnnnagatcggaagagcgtcgtgtagggaaagagtgn

SEQ ID NO: 6 - DNA, 45 bp, Artificial Sequence
  oligo
  modified_base 1: /mod_base="OTHER" /note="5' phosphorylated; a or g or c or t"
  misc_difference 2,3,4,5,6,7,8,9,10,11,12: /note="a or g or c or t"
  modified_base 45: /mod_base="OTHER" /note="3' Inverted dT (reverse linkage)"
nnnnnnnnnnnnagatcggaagagcgtcgtgtagggaaagagtgn

SEQ ID NO: 7 - DNA, 36 bp, Artificial Sequence
  oligo
  modified_base 1: /mod_base="OTHER" /note="5' phosphorylated; a or g or c or t"
  misc_difference 2,3,4,5,6,7,8,9,10,11,12: /note="a or g or c or t"
  modified_base 36: /mod_base="OTHER" /note="3' Inverted dT (reverse linkage)"
nnnnnnnnnnnnagatcggaagagcgtcgtgtaggn

SEQ ID NO: 8 - DNA, 34 bp, Artificial Sequence; identical to SEQ ID NO: 4
  oligo
  modified_base 1: /mod_base="OTHER" /note="5' phosphorylated; a or g or c or t"
  misc_difference 2,3,4,5,6,7,8,9,10: /note="a or g or c or t"
  modified_base 34: /mod_base="OTHER" /note="3' Inverted dT (reverse linkage)"

SEQ ID NO: 9 - DNA, 36 bp, Artificial Sequence; identical to SEQ ID NO: 7
  oligo
  modified_base 1: /mod_base="OTHER" /note="5' phosphorylated; a or g or c or t"
  misc_difference 2,3,4,5,6,7,8,9,10,11,12: /note="a or g or c or t"
  modified_base 36: /mod_base="OTHER" /note="3' Inverted dT (reverse linkage)"

SEQ ID NO: 10 - DNA, 33 bp, Artificial Sequence
  oligo
  modified_base 1: /mod_base="OTHER" /note="5' phosphorylated; a or g or c or t"
  misc_difference 2,3,4,5,6,7,8,9,10,11,12: /note="a or g or c or t"
  modified_base 33: /mod_base="OTHER" /note="g, 3' Spacer C3"
nnnnnnnnnnnntggaattctcgggtgccaagn

SEQ ID NO: 11 - DNA, 53 bp, Artificial Sequence
  oligo
gtgactggagttcagacgtgtgctcttccgatctttttttttttttttttttv

SEQ ID NO: 12 - DNA, 75 bp, Artificial Sequence
  sequencing read
cgatttctaaagggaattcgagctcgcattttgaaaattctatggaagagctagcatctctgacgaaaacagcag

SEQ ID NO: 13 - DNA, 68 bp, Artificial Sequence
  sequencing read
cctttggggaattcgagctcgcattttgaaaattctatggaagagctagcatctctgacgaaaaccag

SEQ ID NO: 14 - DNA, 68 bp, Artificial Sequence
  sequencing read
caaaacgggaattcgagctcgcattttgaaaattctatggaagagctagcatctctgacgaaaacaac

SEQ ID NO: 15 - DNA, 66 bp, Artificial Sequence
  sequencing read
agtggtgggaattcgagctcgcattttgaaaattctatggaagagctagcatctctgacgaaatgc

SEQ ID NO: 16 - DNA, 70 bp, Artificial Sequence
  sequencing read
caaaatgggaattcgagctcgcattttgaaaattctatggaagagctagcatctctgacgaaaacagcgt

SEQ ID NO: 17 - DNA, 65 bp, Artificial Sequence
  sequencing read
tcggacgggaattcgagctcgcattttgaaaattctatggaagagctagcatctcttacgaaaac

SEQ ID NO: 18 - DNA, 66 bp, Artificial Sequence
  sequencing read
ggggacgggaattcgagctcgcattttgaaaattctatggaagagctagcatctctgacaaaaaca

SEQ ID NO: 19 - DNA, 73 bp, Artificial Sequence
  sequencing read
cccgaggggaattcgagctcgcattttgaaaattctatggaagagctagcatctctgacgaaaacggcagaca

SEQ ID NO: 20 - DNA, 71 bp, Artificial Sequence
  sequencing read
aatacagggaattcgagctcgcattttgaaaattctatggaagagctagcatctctgacgaaaacagagag

SEQ ID NO: 21 - DNA, 70 bp, Artificial Sequence; identical to SEQ ID NO: 16
  sequencing read

SEQ ID NO: 22 - DNA, 74 bp, Artificial Sequence
  sequencing read
atttggggaattcgagctcgcattttgaaaattctatggaagagctagcatctctgacgaaaacagcaggcgga

SEQ ID NO: 23 - DNA, 75 bp, Artificial Sequence
  sequencing read
aatggggaattcgagctcgcattttgaaaattctatggaagagctagcatctctgacgaaaacagcaatcggaaa

SEQ ID NO: 24 - DNA, 75 bp, Artificial Sequence
  sequencing read
aaggggaattcgagctcgcattttgaaaattctctggaagagctagcatctctgacgaaaacagcagaacagaaa

SEQ ID NO: 25 - DNA, 75 bp, Artificial Sequence
  sequencing read
ggggaattcgagctcgcattttgaaaatactatggaagagctagcatctctgacgaaaacagcagacgaaaaagt

SEQ ID NO: 26 - DNA, 61 bp, Artificial Sequence
  sequencing read
gggaattcgagctcgcattttgaaaattctatggaagagctagcatctctgactactacag

SEQ ID NO: 27 - DNA, 60 bp, Artificial Sequence
  sequencing read
aagatctcgcattttgaaaattctatggaagagctagcatctctgacgaaaacagcagaa

SEQ ID NO: 28 - DNA, 74 bp, Artificial Sequence
  sequencing read
cgagctcgcattttgaaaattctatggaagagctagcatctctgacgaaaacagcagacggaaaaggagagacc

SEQ ID NO: 29 - DNA, 75 bp, Artificial Sequence
  sequencing read
cgagctcgcattttgaaaattctatggaagagctagcatctctgacgaaaacagcagacggaaaagtactgacca

SEQ ID NO: 30 - DNA, 75 bp, Artificial Sequence
  sequencing read
cgagctcgcattttgaaaattctatggaagagctagcacctctgacgaaaacagcagacggaaaaggactgaaaa

SEQ ID NO: 31 - DNA, 75 bp, Artificial Sequence
  sequencing read
cgagctcgcattttgaaaattctatggaagagctagcatctctgacgaaaacagcagacggaaaagtactgagcc

SEQ ID NO: 32 - DNA, 75 bp, Artificial Sequence; identical to SEQ ID NO: 30
  sequencing read

SEQ ID NO: 33 - DNA, 75 bp, Artificial Sequence
  sequencing read
cgagctcgcattttgaaaattctatggaagagctagcatctctgacgaaaacagcagacggaaaagtactgactc

SEQ ID NO: 34 - DNA, 75 bp, Artificial Sequence; identical to SEQ ID NO: 29
  sequencing read

SEQ ID NO: 35 - DNA, 75 bp, Artificial Sequence
  sequencing read
cgagctcgcattttgaaaattctatggaagagctagcatctctgacgaaaacagcagacggaaaagtacaaaacc

SEQ ID NO: 36 - DNA, 75 bp, Artificial Sequence
  sequencing read
gagctcgcattttgaaaattctatggaagagctagcatctctgacgaaaacagcagacggaaaagtagctgacca

SEQ ID NO: 37 - DNA, 75 bp, Artificial Sequence
  sequencing read
agctcgcattttgaaaattctatggaagagctagcatctctgacgaaaacagcagacggaaaagtactgaccaga

SEQ ID NO: 38 - DNA, 75 bp, Artificial Sequence
  sequencing read
gctcgcattttgaaaattctatggaagagctagcatctctgacgaaaacagcagacggaaaagtacagacccaac

SEQ ID NO: 39 - DNA, 74 bp, Artificial Sequence
  sequencing read
cgcattttgaaaattctatggaagagctagcatctctgacgaaaacagcagacggaaaagtactgaccagctag

SEQ ID NO: 40 - DNA, 73 bp, Artificial Sequence
  sequencing read
cgcattttgaaaattctatggaagagctagcatctctgacgaaaacagcagacggaaaagtactgaccatgca

SEQ ID NO: 41 - DNA, 74 bp, Artificial Sequence
  sequencing read
cgcattttgaaaattctatggaagagctagcatctctgacgaaaacagcagacggaaaagtactgaccagccac

SEQ ID NO: 42 - DNA, 73 bp, Artificial Sequence
  sequencing read
cgcattttgaaaattctatggaagagctagcatctctgacgaaaacagcagacggaaaagtactgaccagcat

SEQ ID NO: 43 - DNA, 129 bp, Artificial Sequence
  consensus sequence
ataaattgagcccgcagcctcccgcttcgctctctgctcctcctgttcgacagtcagccgcatcttcttttgcgtcgccagccgagccacatcgctcagacaccatggggaaggtgaaggtcggagtca

SEQ ID NO: 44 - DNA, 104 bp, Artificial Sequence
  sequencing read
acgtgtgctcgtcactacctccccgggtgctctctgctcctcctgttcgacagtcagccgcatcttcttttgcgtcgccagccgagccacatcgctcagacacc

SEQ ID NO: 45 - DNA, 129 bp, Artificial Sequence
  sequencing read
gaaaattgagcccgcagcctcccgcttcgctctctgctcctcctgttcgacagtcagccgcatcttcttttgcgtcgccagccgagccacatcgctcagacaccatggggaaggtgaaggtcggagtca

SEQ ID NO: 46 - DNA, 122 bp, Artificial Sequence
  sequencing read
aaaatgcattagaggaactgtaaaaatctgctcctccgttcgacagtcagccgcatcttcttttgcgtcgccagccgagccacatcgctcagacaccatggggaaggtgaaggtcggagtca

SEQ ID NO: 47 - DNA, 122 bp, Artificial Sequence
  sequencing read
ctagaggagattggccaacgagattcactggactcctgttcgacagtcagccgcatcttcttttgcgtcgccagccgagccacatcgctgagacaccatggggaaggtgaaggtcggagtca

SEQ ID NO: 48 - DNA, 118 bp, Artificial Sequence
  sequencing read
ttttctgaacgctctggccgctctgctcctcctgttcgacagtcagccgcctcttcgtttgcgtcgccagccgagccacatagctcagacaccaaggggaaggtgaaggtcggagtca

SEQ ID NO: 49 - DNA, 114 bp, Artificial Sequence
  sequencing read
accgagcaccagctttctccgacgccgggaagtcgcagtcagccgcatcttcttttgcgtcgccagccgagccacatcgctcagacaccatggggaaggtgaaggtcggagtca

SEQ ID NO: 50 - DNA, 112 bp, Artificial Sequence
  sequencing read
aacgtgtgctggctctctgctcctcctgttcgacagtcagccgcatcttcttttgcgtcgccagccgagccacatcgctcagacaccatggggaaggtgaaggtcggagtca

SEQ ID NO: 51 - DNA, 110 bp, Artificial Sequence
  sequencing read
ttgctttgggctctctgctcctcctgttcgacagtcagccgcatcttcttttgcgtcgccagccgagccacatcgctcagacaccatggggaaggtgaaggtcggagtca

SEQ ID NO: 52 - DNA, 106 bp, Artificial Sequence
  sequencing read
gatgggctctctgctcctcctgttcgacagtcagccgcatcttcttttgcgtcgccagccgagccacatcgctcagacaccatggggaaggtgaaggtcggagtca

SEQ ID NO: 53 - DNA, 106 bp, Artificial Sequence
  sequencing read
atagggctctctgctcctcctgttcgacagtcagccgcatcttcttttgcgtcgccagccgagccacatcgctcagacaccatggggaaggcgaaggtcggagtca

SEQ ID NO: 54 - DNA, 106 bp, Artificial Sequence
  sequencing read
atctggctctctgctcctcctgttcgacagtcagccgcatcttcttttgcgtcgccagccgagccacatcgctgagacaccatggggaaggtgaaggtcggagtca

SEQ ID NO: 55 - DNA, 106 bp, Artificial Sequence
  sequencing read
acgtggctctctgctcctcctgttcgacagtcagccgcatcttcttttgcgtcgccagccgagccacatcgctcagacaccatggggaaggtgaaggtcggagtca

SEQ ID NO: 56 - DNA, 106 bp, Artificial Sequence; identical to SEQ ID NO: 55
  sequencing read

SEQ ID NO: 57 - DNA, 97 bp, Artificial Sequence
  sequencing read
ttgcggctctctgctcctcctgttcgacagtcagccgcatcttcttttgcgtcgccagccgagccacatcgctcagacaccatggggaagcggaaca

SEQ ID NO: 58 - DNA, 82 bp, Artificial Sequence
  sequencing read
gggggctctctgctcctcctgttcgacagtcagccgcatcttcttttgcgtcgccagccgagccacatcgctcagaccccac

SEQ ID NO: 59 - DNA, 105 bp, Artificial Sequence
  sequencing read
aatggctctctgctcctcctgttcgacagtcagccgcatcttcttttgcgtcgccagccgagccacatcgctcagacaccatggggaaggtgaaggtcggagtca

SEQ ID NO: 60 - DNA, 105 bp, Artificial Sequence
  sequencing read
atcggctctctgctcctcctgttcgacagtcagccgcatcttcttttgcgtcgccagccgagccacatcgctcagacaccatggggaaggtgaaggtcggagtca

SEQ ID NO: 61 - DNA, 105 bp, Artificial Sequence
  sequencing read
attggctctctgctcctcctgttcgacagtcagccgcatcttcttttgcgtcgccagccgagccacatcgctcagacaccatggggaaggtgaaggtcggagtca

SEQ ID NO: 62 - DNA, 57 bp, Artificial Sequence
  sequencing read
gttggctctctgctcctcctgttcgacagtcagccgcatcttcttttgcaatcgcca

SEQ ID NO: 63 - DNA, 104 bp, Artificial Sequence
  sequencing read
atggctctctgctcctcctgttcgacagtcagccgcatcttcttttgcgtcgccagccgagccacatcgctcagacaccatggggaaggtgaaggtcggagtca

SEQ ID NO: 64 - DNA, 104 bp, Artificial Sequence
  sequencing read
ttggctctctgctcctcctgttcgacagtcagccgcatcttcttttgcgtcgccagccgagccacatcgctcagacaccatggggaaggtgaaggtcggagtca

SEQ ID NO: 65 - DNA, 82 bp, Artificial Sequence
  sequencing read
ggggctctctgctcctcctgttcgacagtcagccgcatcttcttttgcgtcgccagccgagccacatcgctcagaacagcca

SEQ ID NO: 66 - DNA, 104 bp, Artificial Sequence
  sequencing read
gtggctctctgctcctcctgttcgacagtcagccgcatcttcctttgcgtcgccagccgagccacatcgctcagacaccatggggaaggtgaaggtcggagtca

SEQ ID NO: 67 - DNA, 103 bp, Artificial Sequence
  sequencing read
gggctctctgctcctcctgttcgacagtcagccgcatcttcttttgcgtcgccagccgagccacatcgctcagacaccatggggaaggtgaaggtcggagtca